European Patent Application EP 4 137 209 A1, published February 22, 2023. Title: TFF2蛋白和IFN-κ蛋白联用在治疗新型冠状病毒感染中的应用. Applicant: 上海市公共卫生临床中心. The sequence listing filed with the application follows.

SEQUENCE LISTING (16 sequences)

SEQ ID NO: 1 - protein, 107 aa, 人工序列
MEKPSPCQCSRLSPHNRTNCGFPGITSDQCFDNGCCFDSSVTGVPWCFHPLPKQESDQCVMEVSDRRNCGYPGISPEECASRKCCFSNFIFEVPWCFFPKSVEDCHY

SEQ ID NO: 2 - protein, 107 aa, 人工序列
MEKPSPCRCSRLTPHNRKNCGFPGITSEQCFDLGCCFDSSVAGVPWCFHPLPNQESEQCVMEVSARKNCGYPGISPEDCASRNCCFSNLIFEVPWCFFPQSVEDCHY

SEQ ID NO: 3 - DNA, 603 bp, 智人（Homo sapiens）
attctgcaagccaccctggggtgcagctgagctagacatgggacggcgagacgcccagctcctggcagcgctcctcgtcctggggctatgtgccctggcggggagtgagaaaccctccccctgccagtgctccaggctgagcccccataacaggacgaactgcggcttccctggaatcaccagtgaccagtgttttgacaatggatgctgtttcgactccagtgtcactggggtcccctggtgtttccaccccctcccaaagcaagagtcggatcagtgcgtcatggaggtctcagaccgaagaaactgtggctacccgggcatcagccccgaggaatgcgcctctcggaagtgctgcttctccaacttcatctttgaagtgccctggtgcttcttcccgaagtctgtggaagactgccattactaagagaggctggttccagaggatgcatctggctcaccgggtgttccgaaaccaaagaagaaacttcgccttatcagcttcatacttcatgaaatcctgggttttcttaaccatcttttcctcattttcaatggtttaacatataatttctttaaataaaacccttaaaatctgctaaa

SEQ ID NO: 4 - DNA, 390 bp, 智人（Homo sapiens）
atgggacggcgagacgcccagctcctggcagcgctcctcgtcctggggctatgtgccctggcggggagtgagaaaccctccccctgccagtgctccaggctgagcccccataacaggacgaactgcggcttccctggaatcaccagtgaccagtgttttgacaatggatgctgtttcgactccagtgtcactggggtcccctggtgtttccaccccctcccaaagcaagagtcggatcagtgcgtcatggaggtctcagaccgaagaaactgtggctacccgggcatcagccccgaggaatgcgcctctcggaagtgctgcttctccaacttcatctttgaagtgccctggtgcttcttcccgaagtctgtggaagactgccattactaa

SEQ ID NO: 5 - DNA, 571 bp, 小鼠（Mus musculus）
attctgcaggctgcccaggtccagtggagcagacatgcgacctcgaggtgcccccctgctggcagtggtcctggttttgggactgcatgctctggtagagggcgagaaaccttccccctgtcggtgctccaggctgacaccccacaacagaaagaactgtggcttcccgggcatcaccagtgagcagtgctttgatcttggatgctgctttgactctagcgtcgctggggtcccttggtgtttccacccacttccaaaccaagaatcggagcagtgtgtcatggaagtgtcagctcgcaagaattgtgggtacccgggcatcagtcccgaggactgtgccagtcgaaactgctgcttttccaacctgatctttgaagtgccctggtgtttcttcccacagtctgtggaagattgtcactactgagagttgctactgccgagccacccgttccctgggagctgcaagccagaagaaagtttcaaccagacttcatcaatctctggggtttctaaaaccatcttgacccttagcagtggctagacacagcattttccaagtaaagaaaagttg

SEQ ID NO: 6 - DNA, 390 bp, 小鼠（Mus musculus）
atgcgacctcgaggtgcccccctgctggcagtggtcctggttttgggactgcatgctctggtagagggcgagaaaccttccccctgtcggtgctccaggctgacaccccacaacagaaagaactgtggcttcccgggcatcaccagtgagcagtgctttgatcttggatgctgctttgactctagcgtcgctggggtcccttggtgtttccacccacttccaaaccaagaatcggagcagtgtgtcatggaagtgtcagctcgcaagaattgtgggtacccgggcatcagtcccgaggactgtgccagtcgaaactgctgcttttccaacctgatctttgaagtgccctggtgtttcttcccacagtctgtggaagattgtcactactga

SEQ ID NO: 7 - protein, 181 aa, 人工序列
MLDCNLLNVHLRRVTWQNLRHLSSMSNSFPVECLRENIAFELPQEFLQYTQPMKRDIKKAFYEMSLQAFNIFSQHTFKYWKERHLKQIQIGLDQQAEYLNQCLEEDKNENEDMKEMKENEMKPSEARVPQLSSLELRRYFHRIDNFLKEKKYSDCAWEIVRVEIRRCLYYFYKFTALFRRK

SEQ ID NO: 8 - protein, 179 aa, 人工序列
MLNCVYLDDSILENVKLLGSTMTGFPLRCLKDITDFKFPKEILPYIQHMKREINAVSYRISSLALTIFNLKGSIPPVTEEHWERIRSGLFKQVRQAQECFMDEEKENREHPHSEDFLTVYLELGKYFFRIKKFLINKKYSFCAWKIVTVEIRRCFIIFSKSRKLLKMISESPTFKQELK

SEQ ID NO: 9 - DNA, 1140 bp, 智人（Homo sapiens）
ggattttttagcttgcaaaaaaaatgagcaccaaacctgatatgattcaaaagtgtttgtggcttgagatccttatgggtatattcattgctggcaccctatccctggactgtaacttactgaacgttcacctgagaagagtcacctggcaaaatctgagacatctgagtagtatgagcaattcatttcctgtagaatgtctacgagaaaacatagcttttgagttgccccaagagtttctgcaatacacccaacctatgaagagggacatcaagaaggccttctatgaaatgtccctacaggccttcaacatcttcagccaacacaccttcaaatattggaaagagagacacctcaaacaaatccaaataggacttgatcagcaagcagagtacctgaaccaatgcttggaggaagacaagaatgaaaatgaagacatgaaagaaatgaaagagaatgagatgaaaccctcagaagccagggtcccccagctgagcagcctggaactgaggagatatttccacaggatagacaatttcctgaaagaaaagaaatacagtgactgtgcctgggagattgtccgagtggaaatcagaagatgtttgtattacttttacaaatttacagctctattcaggaggaaataagaatcatctaccttcaagcaagaattaacagagattgtggctacgcaaatgcaccaaaaaagggtgaaatatatctgaaatgtacctggttctgcccttggaagccatttcctgctcatgccactaacagcatgctgccaaactgttcagattcaagattattccaagcgcagggcccaaatgttatagccaaagaaagtcttatgataaaagtgaggcaaatttcagccaagaagttagaagagatgtttaaaagaacaagaacaaattgtggatcatggtatatgcaggctatcagcagaaggatcagacaataaaatgagttagtgcaaaccatttagtaaaaataactatcagcagagttgttccagattaaaaatagtactacaagcttgtaaaggagttaggacatgcaagctactgagcataaaatatatacttgctatttttcatgactttctctaataaagtctttgcctgttctctctaataa

SEQ ID NO: 10 - DNA, 624 bp, 智人（Homo sapiens）
atgagcaccaaacctgatatgattcaaaagtgtttgtggcttgagatccttatgggtatattcattgctggcaccctatccctggactgtaacttactgaacgttcacctgagaagagtcacctggcaaaatctgagacatctgagtagtatgagcaattcatttcctgtagaatgtctacgagaaaacatagcttttgagttgccccaagagtttctgcaatacacccaacctatgaagagggacatcaagaaggccttctatgaaatgtccctacaggccttcaacatcttcagccaacacaccttcaaatattggaaagagagacacctcaaacaaatccaaataggacttgatcagcaagcagagtacctgaaccaatgcttggaggaagacaagaatgaaaatgaagacatgaaagaaatgaaagagaatgagatgaaaccctcagaagccagggtcccccagctgagcagcctggaactgaggagatatttccacaggatagacaatttcctgaaagaaaagaaatacagtgactgtgcctgggagattgtccgagtggaaatcagaagatgtttgtattacttttacaaatttacagctctattcaggaggaaataa

SEQ ID NO: 11 - DNA, 872 bp, 小鼠（Mus musculus）
ctaagcaccagggttgagaatgactccaaagtttttatggctggtggcccttgtggctctatacattccgcccatccaatctctgaactgtgtttacctggatgatagcatcttggaaaatgtgaaacttctgggcagtaccatgaccggctttcccttaagatgtctaaaagatatcacagattttaagtttcctaaagagattttgccatacatccagcatatgaaaagggagataaacgccgtctcctatcgtatatcctctctggcactaactatcttcaatcttaaaggctccatccctccagtgacagaggaacactgggaacgtatcagatcgggacttttcaaacaagtgcggcaagctcaagagtgcttcatggacgaggagaaagagaacagggaacatcctcactccgaggacttcctgacagtctacctggagttgggcaagtatttcttcagaatcaaaaagttcctgataaataagaaatacagtttctgtgcatggaagattgtcacagtggaaataagaagatgtttcattatattttccaagtccagaaaactactcaaaatgatatcagaatcacccaccttcaagcaagaacttaaatagaagctgcaattgctcaaatgtctccaagaacgctttattctaaagccattaccaggatgctgctaatgctaccttcagatgcaagacttttcaagttcagggttcaaggcagtgcagtcaaagaaagtcttaagcaaaagatgaacttcagtggaaaagttagcagaaatgttaacttataataaaaccaaagttatacataaaaaaaaaaaaaaaaaaaaaaaaaaaaaaaaaaaaaaaaaaaaaaaaaaaa

SEQ ID NO: 12 - DNA, 600 bp, 小鼠（Mus musculus）
atgactccaaagtttttatggctggtggcccttgtggctctatacattccgcccatccaatctctgaactgtgtttacctggatgatagcatcttggaaaatgtgaaacttctgggcagtaccatgaccggctttcccttaagatgtctaaaagatatcacagattttaagtttcctaaagagattttgccatacatccagcatatgaaaagggagataaacgccgtctcctatcgtatatcctctctggcactaactatcttcaatcttaaaggctccatccctccagtgacagaggaacactgggaacgtatcagatcgggacttttcaaacaagtgcggcaagctcaagagtgcttcatggacgaggagaaagagaacagggaacatcctcactccgaggacttcctgacagtctacctggagttgggcaagtatttcttcagaatcaaaaagttcctgataaataagaaatacagtttctgtgcatggaagattgtcacagtggaaataagaagatgtttcattatattttccaagtccagaaaactactcaaaatgatatcagaatcacccaccttcaagcaagaacttaaatag

SEQ ID NO: 13 - DNA, 29 bp, 人工序列
cgctctagaatgcgacctcgaggtgcccc

SEQ ID NO: 14 - DNA, 29 bp, 人工序列
cctggatcctcagtagtgacaatcttcca

SEQ ID NO: 15 - DNA, 25 bp, 人工序列
cgctctagaatgagcaccaaacctg

SEQ ID NO: 16 - DNA, 24 bp, 人工序列
tctggatccttatttcctcctgaa